European Patent Application EP 4 311 559 A1, published January 31, 2024. Title: NANOPARTICLES AND PEPTIDES FOR THE DELIVERY OF CARGOS TO CHONDROCYTES. Applicant: 4basebio UK Ltd. Application EP. The sequence listing filed with the application follows.

SEQUENCE LISTING (40 sequences)

SEQ ID NO: 1 - protein, 7 aa, synthetic construct
STLHQKL

SEQ ID NO: 2 - protein, 7 aa, synthetic construct
SSLHQKL

SEQ ID NO: 3 - protein, 12 aa, synthetic construct
RLDPTSYLRTFW

SEQ ID NO: 4 - protein, 12 aa, synthetic construct
HDSQLEALIKFM

SEQ ID NO: 5 - protein, 12 aa, synthetic construct
DWRVIIPPRPSA

SEQ ID NO: 6 - protein, 9 aa, synthetic construct
GASTLHQKL

SEQ ID NO: 7 - protein, 11 aa, synthetic construct
GACSTLHQKLC

SEQ ID NO: 8 - protein, 15 aa, synthetic construct
GARVRRCSTLHQKLC

SEQ ID NO: 9 - protein, 25 aa, synthetic construct
KKKKKKKKKKKKKKKKGASTLHQKL

SEQ ID NO: 10 - protein, 27 aa, synthetic construct
KKKKKKKKKKKKKKKKGACSTLHQKLC

SEQ ID NO: 11 - protein, 31 aa, synthetic construct
KKKKKKKKKKKKKKKKGARVRRCSTLHQKLC

SEQ ID NO: 12 - protein, 9 aa, synthetic construct
GASSLHQKL

SEQ ID NO: 13 - protein, 11 aa, synthetic construct
GACSSLHQKLC

SEQ ID NO: 14 - protein, 15 aa, synthetic construct
GARVRRCSSLHQKLC

SEQ ID NO: 15 - protein, 25 aa, synthetic construct
KKKKKKKKKKKKKKKKGASSLHQKL

SEQ ID NO: 16 - protein, 27 aa, synthetic construct
KKKKKKKKKKKKKKKKGACSSLHQKLC

SEQ ID NO: 17 - protein, 31 aa, synthetic construct
KKKKKKKKKKKKKKKKGARVRRCSSLHQKLC

SEQ ID NO: 18 - protein, 14 aa, synthetic construct
GARLDPTSYLRTFW

SEQ ID NO: 19 - protein, 16 aa, synthetic construct
GACRLDPTSYLRTFWC

SEQ ID NO: 20 - protein, 20 aa, synthetic construct
GARVRRCRLDPTSYLRTFWC

SEQ ID NO: 21 - protein, 30 aa, synthetic construct
KKKKKKKKKKKKKKKKGARLDPTSYLRTFW

SEQ ID NO: 22 - protein, 32 aa, synthetic construct
KKKKKKKKKKKKKKKKGACRLDPTSYLRTFWC

SEQ ID NO: 23 - protein, 36 aa, synthetic construct
KKKKKKKKKKKKKKKKGARVRRCRLDPTSYLRTFWC

SEQ ID NO: 24 - protein, 14 aa, synthetic construct
GAHDSQLEALIKFM

SEQ ID NO: 25 - protein, 16 aa, synthetic construct
GACHDSQLEALIKFMC

SEQ ID NO: 26 - protein, 20 aa, synthetic construct
RVRRGACHDSQLEALIKFMC

SEQ ID NO: 27 - protein, 30 aa, synthetic construct
KKKKKKKKKKKKKKKKGAHDSQLEALIKFM

SEQ ID NO: 28 - protein, 32 aa, synthetic construct
KKKKKKKKKKKKKKKKGACHDSQLEALIKFMC

SEQ ID NO: 29 - protein, 36 aa, synthetic construct
KKKKKKKKKKKKKKKKRVRRGACHDSQLEALIKFMC

SEQ ID NO: 30 - protein, 14 aa, synthetic construct
GADWRVIIPPRPSA

SEQ ID NO: 31 - protein, 16 aa, synthetic construct
GACDWRVIIPPRPSAC

SEQ ID NO: 32 - protein, 20 aa, synthetic construct
RVRRGACDWRVIIPPRPSAC

SEQ ID NO: 33 - protein, 18 aa, synthetic construct
RVRRCDWRVIIPPRPSAC

SEQ ID NO: 34 - protein, 30 aa, synthetic construct
KKKKKKKKKKKKKKKKGADWRVIIPPRPSA

SEQ ID NO: 35 - protein, 32 aa, synthetic construct
KKKKKKKKKKKKKKKKGACDWRVIIPPRPSAC

SEQ ID NO: 36 - protein, 34 aa, synthetic construct
KKKKKKKKKKKKKKKKRVRRCDWRVIIPPRPSAC

SEQ ID NO: 37 - protein, 36 aa, synthetic construct
KKKKKKKKKKKKKKKKRVRRGACDWRVIIPPRPSAC

SEQ ID NO: 38 - protein, 9 aa, synthetic construct
CSTLKQKLC

SEQ ID NO: 39 - protein, 4 aa, synthetic construct
RVRR

SEQ ID NO: 40 - DNA, 13 bp, synthetic construct
  source 1..13: mol_type = other DNA
aaaaaacataaaa